European Patent Application EP 4 201 415 A1, published June 28, 2023. Title: Faecalibacterium prausnitzii strain and uses thereof. Applicant: KoBioLabs, Inc. The sequence listing filed with the application follows.

SEQUENCE LISTING (14 sequences)

SEQ ID NO: 1 - DNA, 20 bp, Artificial Sequence
  (synthetic) 27F primer
  misc_feature (11): y is t or c
  misc_feature (12): m is a or c
agagtttgatymtggctcag

SEQ ID NO: 2 - DNA, 21 bp, Artificial Sequence
  (synthetic) 1492R primer
  misc_feature (6): y is t or c
tacggytaccttgttacgact

SEQ ID NO: 3 - DNA, 1383 bp, Faecalibacterium prausnitzii
gacgaacgctggcggcgcgcctaacacatgcaagtcgaacgagtgagagagagcttgctttctcgagcgagtggcgaacgggtgagtaacgcgtgaggaacctgcctcaaagagggggacaacagttggaaacgactgctaataccgcataagcccacgacccggcatcgggtagagggaaaaggagcaatccgctttgagatggcctcgcgtccgattagctagttggtgaggtaactggcccaccaaggcgacgatcggtagccggactgagaggttgaacggccacattgggactgagacacggcccagactcctacgggaggcagcagtggggaatattgcacaatgggggaaaccctgatgcagcgacgccgcgtggaggaagaaggtcttcggattgtaaactcctgttgttgaggaagataatgacggtactcaacaaggaagtgacggctaactacgtgccagcagccgcggtaaaacgtaggtcacaagcgttgtccggaattactgggtgtaaagggagcgcaggcgggaagacaagttggaagtgaaatccatgggctcaacccatgaactgctttcaaaactgtttttcttgagtagtgcagaggtaggcggaattcccggtgtagcggtggaatgcgtagatatcgggaggaacaccagtggcgaaggcggcctactgggcaccaactgacgctgaggctcgaaagtgtgggtagcaaacaggattagataccctggtagtccacactgtaaacgatgattactaggtgttggaggattgaccccttcagtgccgcagttaacacaataagtaatccacctggggagtacgaccgcaaggttgaaactcaaaggaattgacgggggcccgcacaagcagtggagtatgtggtttaattcgacgcaacgcgaagaaccttaccaagtcttgacatcctgcgacgcacatagaaacagtagtttccttcgggacgcagagacaggtggtgcatggttgtcgtcagctcgtgtcgtgagatgttgggttaagtcccgcaacgagcgcaacccttatggtcagttactacgcaagaggactctggccagactgccgttgacaaaacggaggaaggtggggatgacgtcaaatcatcatgccctttatgacttgggctacacacgtactacaatggcgttaaacaaagagaagcaagaccgcgaggtggagcaaaactcagaaacaacgtcccagttcggactgcaggctgcaactcgcctgcacgaagtcggaattgctagtaatcgcagatcagcatgctgcggtgaatacgttcccgggccttgtacacaccgcccgtcacaccatgagagccggggggacccgaagtcggt

SEQ ID NO: 4 - DNA, 1414 bp, Faecalibacterium prausnitzii
tgaatttggctcaggacgaacgctggcggcgcgcctaacacatgcaagtcgaacgagcgagagagagcttgctttctcagagcgagtggcgaacgggtgagtaacgcgtgaggaacctgcctcaaagagggggacaacagttggaaacgactgctaataccgcataagcccacgacccggcatcgggtagagggaaaaggagcaatccgctttgagatggcctcgcgtccgattagctagttggtgaggtaacggcccaccaaggcgacgatcggtagccggactgagaggttgaacggccacattgggactgagacacggcccagactcctacgggaggcagcagtggggaatattgcacaatgggggaaaccctgatgcagcgacgccgcgtggaggaagaaggtcttcggattgtaaactcctgttgttgaggaagataatgacggtactcaacaaggaagtgacggctaactacgtgccagcagccgcggtaaaacgtaggtcacaagcgttgtccggaattactgggtgtaaagggagcgcaggcgggaagacaagttggaagtgaaatccatgggctcaacccatgaactgctttcaaaactgtttttcttgagtagtgcagaggtaggcggaattcccggtgtagcggtggaatgcgtagatatcgggaggaacaccagtggcgaaggcggcctactgggcaccaactgacgctgaggctcgaaagtgtgggtagcaaacaggattagataccctggtagtccacactgtaaacgatgattactaggggttggaggattgaccccttcagtgccgcagttaacacaataagtaatccacctggggagtacgaccgcaaggttgaaactcaaaggaattgacgggggcccgcacaagcagtggagtatgtggtttaattcgacgcaacgcgaagaaccttaccaagtcttgacatcctgcgacgcacatagaaatatgtgtttccttcgggacgcagagacaggtggtgcatggttgtcgtcagctcgtgtcgtgagatgttgggttaagtcccgcaacgagcgcaacccttatggtcagttactacgcaagaggactctggccagactgccgttgacaaaacggaggaaggtggggatgacgtcaaatcatcatgccctttatgacttgggctacacacgtactacaatggcgttaaacaaagagaagcaagaccgcgaggtggagcaaaactcagaaacaacgtcccagttcggactgcaggctgcaactcgcctgcacgaagtcggaattgctagtaatcgcagatcagcatgctgcggtgaatacgttcccgggccttgtacacaccgcccgtcacaccatgagagccggggggacccgaagtcggtagtctaaccgcaaggag

SEQ ID NO: 5 - DNA, 59 bp, Artificial Sequence
  (synthetic) 515F primer
  misc_feature (49): m is a or c
atgatacggcgaccaccgagatctacactatggtaattgtgtgccagcmgccgcggtaa

SEQ ID NO: 6 - DNA, 56 bp, Artificial Sequence
  (synthetic) 806R primer
  misc_feature (44): h is a, c, or t
  misc_feature (45): v is g, c, or a
  misc_feature (50): w is a or t
caagcagaagacggcatacgagatagtcagtcagccggactachvgggtwtctaat

SEQ ID NO: 7 - DNA, 21 bp, Artificial Sequence
  (synthetic) HPRT primer FWD
ttatggacaggactgaaagac

SEQ ID NO: 8 - DNA, 22 bp, Artificial Sequence
  (synthetic) HPRT primer RVS
gctttaatgtaatccagcaggt

SEQ ID NO: 9 - DNA, 20 bp, Artificial Sequence
  (synthetic) IL-10 primer FWD
ataactgcacccacttccca

SEQ ID NO: 10 - DNA, 20 bp, Artificial Sequence
  (synthetic) IL-10 primer RVS
tcatttccgataaggcttgg

SEQ ID NO: 11 - DNA, 24 bp, Artificial Sequence
  (synthetic) Zo-1 primer FWD
acccgaaactgatgctgtggatag

SEQ ID NO: 12 - DNA, 24 bp, Artificial Sequence
  (synthetic) Zo-1 primer RVS
aaatggccgggcagaacttgtgta

SEQ ID NO: 13 - DNA, 21 bp, Artificial Sequence
  (synthetic) Occludin primer FWD
ggaggactgggtcagggaata

SEQ ID NO: 14 - DNA, 20 bp, Artificial Sequence
  (synthetic) Occludin primer RVS
cgtcgtctagttctgcctgt